European Patent Specification EP 4 626 447 B1, published September 16, 2026. Title: BISPECIFIC CHIMERIC ANTIGEN RECEPTORS TARGETING CD20 AND BCMA. Applicant: ABELZETA INC. The sequence listing filed with the application follows.

SEQUENCE LISTING (146 sequences)

SEQ ID NO: 1 - DNA, 63 bp, synthetic construct
  source 1..63: mol_type = other DNA
atggccttaccagtgaccgccttgctcctgccgctggccttgctgctccacgccgccaggccg

SEQ ID NO: 2 - protein, 21 aa, synthetic construct
MALPVTALLLPLALLLHAARP

SEQ ID NO: 3 - DNA, 321 bp, synthetic construct
  source 1..321: mol_type = other DNA
gaaattgtgttgacacagtctccagccaccctgtctttgtctccaggggaaagagccaccctctcctgcagggccagtcagagtgttagcagctacttagcctggtaccaacagaaacctggccaggctcccaggctcctcatctatgatgcatccaacagggccactggcatcccagccaggttcagtggcagtgggtctgggacagacttcactctcaccatcagcagcctagagcctgaagattttgcagtttattactgtcagcagcgtagcaactggccgatcaccttcggccaagggacacgactggagattaaa

SEQ ID NO: 4 - protein, 107 aa, synthetic construct
EIVLTQSPATLSLSPGERATLSCRASQSVSSYLAWYQQKPGQAPRLLIYDASNRATGIPARFSGSGSGTDFTLTISSLEPEDFAVYYCQQRSNWPITFGQGTRLEIK

SEQ ID NO: 5 - DNA, 54 bp, synthetic construct
  source 1..54: mol_type = other DNA
ggcagtactagcggtggtggctccgggggcggttccggtgggggcggcagcagc

SEQ ID NO: 6 - protein, 18 aa, synthetic construct
GSTSGGGSGGGSGGGGSS

SEQ ID NO: 7 - DNA, 366 bp, synthetic construct
  source 1..366: mol_type = other DNA
gaagtgcagctggtggagtctgggggaggcttggtacagcctggcaggtccctgagactctcctgtgcagcctctggattcacctttaatgattatgccatgcactgggtccggcaagctccagggaagggcctggagtgggtctcaactattagttggaatagtggttccataggctatgcggactctgtgaagggccgattcaccatctccagagacaacgccaagaagtccctgtatctgcaaatgaacagtctgagagctgaggacacggccttgtattactgtgcaaaagatatacagtacggcaactactactacggtatggacgtctggggccaagggaccacggtcaccgtctcctca

SEQ ID NO: 8 - protein, 122 aa, synthetic construct
EVQLVESGGGLVQPGRSLRLSCAASGFTFNDYAMHWVRQAPGKGLEWVSTISWNSGSIGYADSVKGRFTISRDNAKKSLYLQMNSLRAEDTALYYCAKDIQYGNYYYGMDVWGQGTTVTVSS

SEQ ID NO: 9 - DNA, 15 bp, synthetic construct
  source 1..15: mol_type = other DNA
ggaggtggtggatcc

SEQ ID NO: 10 - protein, 5 aa, synthetic construct
GGGGS

SEQ ID NO: 11 - DNA, 321 bp, synthetic construct
  source 1..321: mol_type = other DNA
gacatccagatgacccagtccccctcctccctgtccgcctccgtgggcgaccgggtgaccatcacctgccgggcctcccagggcatctccaactacctgaactggtaccagcagaagcccggcaaggcccccaagcccctgatctactacacctccaacctgcagtccggcgtgccctcccggttctccggctccggctccggcaccgactacaccctgaccatctcctccctgcagcccgaggacttcgccacctactactgcatgggccagaccatctcctcctacaccttcggccagggcaccaagctggagatcaag

SEQ ID NO: 12 - protein, 107 aa, synthetic construct
DIQMTQSPSSLSASVGDRVTITCRASQGISNYLNWYQQKPGKAPKPLIYYTSNLQSGVPSRFSGSGSGTDYTLTISSLQPEDFATYYCMGQTISSYTFGQGTKLEIK

SEQ ID NO: 13 - DNA, 45 bp, synthetic construct
  source 1..45: mol_type = other DNA
ggtggcggtggctcgggcggtggtgggtcgggtggcggcggatct

SEQ ID NO: 14 - protein, 15 aa, synthetic construct
GGGGSGGGGSGGGGS

SEQ ID NO: 15 - DNA, 363 bp, synthetic construct
  source 1..363: mol_type = other DNA
gaggtgcagctggtggagtccggcggcggcctggtgcagcccggcggctccctgcggctgtcctgcgccgcctccggcttcaccttctccaacttcgacatggcctgggtgcggcaggcccccggcaagggcctggtgtgggtgtcctccatcaccaccggcgccgaccacgccatctacgccgactccgtgaagggccggttcaccatctcccgggacaacgccaagaacaccctgtacctgcagatgaactccctgcgggccgaggacaccgccgtgtactactgcgtgcggcacggctactacgacggctaccacctgttcgactactggggccagggcaccctggtgaccgtgtcctcc

SEQ ID NO: 16 - protein, 121 aa, synthetic construct
EVQLVESGGGLVQPGGSLRLSCAASGFTFSNFDMAWVRQAPGKGLVWVSSITTGADHAIYADSVKGRFTISRDNAKNTLYLQMNSLRAEDTAVYYCVRHGYYDGYHLFDYWGQGTLVTVSS

SEQ ID NO: 17 - DNA, 165 bp, synthetic construct
  source 1..165: mol_type = other DNA
ttcgtgccggtcttcctgccagcgaagcccaccacgacgccagcgccgcgaccaccaacaccggcgcccaccatcgcgtcgcagcccctgtccctgcgcccagaggcgtgccggccagcggcggggggcgcagtgcacacgagggggctggacttcgcctgtgat

SEQ ID NO: 18 - protein, 55 aa, synthetic construct
FVPVFLPAKPTTTPAPRPPTPAPTIASQPLSLRPEACRPAAGGAVHTRGLDFACD

SEQ ID NO: 19 - DNA, 72 bp, synthetic construct
  source 1..72: mol_type = other DNA
atctacatctgggcgcccttggccgggacttgtggggtccttctcctgtcactggttatcaccctttactgc

SEQ ID NO: 20 - protein, 24 aa, synthetic construct
IYIWAPLAGTCGVLLLSLVITLYC

SEQ ID NO: 21 - DNA, 126 bp, synthetic construct
  source 1..126: mol_type = other DNA
aaacggggcagaaagaaactcctgtatatattcaaacaaccatttatgagaccagtacaaactactcaagaggaagatggctgtagctgccgatttccagaagaagaagaaggaggatgtgaactg

SEQ ID NO: 22 - protein, 42 aa, synthetic construct
KRGRKKLLYIFKQPFMRPVQTTQEEDGCSCRFPEEEEGGCEL

SEQ ID NO: 23 - DNA, 339 bp, synthetic construct
  source 1..339: mol_type = other DNA
agagtgaagttcagcaggagcgcagacgcccccgcgtaccagcagggccagaaccagctctataacgagctcaatctaggacgaagagaggagtacgatgttttggacaagagacgtggccgggaccctgagatggggggaaagccgagaaggaagaaccctcaggaaggcctgtacaatgaactgcagaaagataagatggcggaggcctacagtgagattgggatgaaaggcgagcgccggaggggcaaggggcacgatggcctttaccagggtctcagtacagccaccaaggacacctacgacgcccttcacatgcaggccctgccccctcgctaa

SEQ ID NO: 24 - protein, 112 aa, synthetic construct
RVKFSRSADAPAYQQGQNQLYNELNLGRREEYDVLDKRRGRDPEMGGKPRRKNPQEGLYNELQKDKMAEAYSEIGMKGERRRGKGHDGLYQGLSTATKDTYDALHMQALPPR

SEQ ID NO: 25 - DNA, 2250 bp, synthetic construct
  source 1..2250: mol_type = other DNA
atggccttaccagtgaccgccttgctcctgccgctggccttgctgctccacgccgccaggccggaaattgtgttgacacagtctccagccaccctgtctttgtctccaggggaaagagccaccctctcctgcagggccagtcagagtgttagcagctacttagcctggtaccaacagaaacctggccaggctcccaggctcctcatctatgatgcatccaacagggccactggcatcccagccaggttcagtggcagtgggtctgggacagacttcactctcaccatcagcagcctagagcctgaagattttgcagtttattactgtcagcagcgtagcaactggccgatcaccttcggccaagggacacgactggagattaaaggcagtactagcggtggtggctccgggggcggttccggtgggggcggcagcagcgaagtgcagctggtggagtctgggggaggcttggtacagcctggcaggtccctgagactctcctgtgcagcctctggattcacctttaatgattatgccatgcactgggtccggcaagctccagggaagggcctggagtgggtctcaactattagttggaatagtggttccataggctatgcggactctgtgaagggccgattcaccatctccagagacaacgccaagaagtccctgtatctgcaaatgaacagtctgagagctgaggacacggccttgtattactgtgcaaaagatatacagtacggcaactactactacggtatggacgtctggggccaagggaccacggtcaccgtctcctcaggaggtggtggatccgacatccagatgacccagtccccctcctccctgtccgcctccgtgggcgaccgggtgaccatcacctgccgggcctcccagggcatctccaactacctgaactggtaccagcagaagcccggcaaggcccccaagcccctgatctactacacctccaacctgcagtccggcgtgccctcccggttctccggctccggctccggcaccgactacaccctgaccatctcctccctgcagcccgaggacttcgccacctactactgcatgggccagaccatctcctcctacaccttcggccagggcaccaagctggagatcaagggtggcggtggctcgggcggtggtgggtcgggtggcggcggatctgaggtgcagctggtggagtccggcggcggcctggtgcagcccggcggctccctgcggctgtcctgcgccgcctccggcttcaccttctccaacttcgacatggcctgggtgcggcaggcccccggcaagggcctggtgtgggtgtcctccatcaccaccggcgccgaccacgccatctacgccgactccgtgaagggccggttcaccatctcccgggacaacgccaagaacaccctgtacctgcagatgaactccctgcgggccgaggacaccgccgtgtactactgcgtgcggcacggctactacgacggctaccacctgttcgactactggggccagggcaccctggtgaccgtgtcctccttcgtgccggtcttcctgccagcgaagcccaccacgacgccagcgccgcgaccaccaacaccggcgcccaccatcgcgtcgcagcccctgtccctgcgcccagaggcgtgccggccagcggcggggggcgcagtgcacacgagggggctggacttcgcctgtgatatctacatctgggcgcccttggccgggacttgtggggtccttctcctgtcactggttatcaccctttactgcaaacggggcagaaagaaactcctgtatatattcaaacaaccatttatgagaccagtacaaactactcaagaggaagatggctgtagctgccgatttccagaagaagaagaaggaggatgtgaactgagagtgaagttcagcaggagcgcagacgcccccgcgtaccagcagggccagaaccagctctataacgagctcaatctaggacgaagagaggagtacgatgttttggacaagagacgtggccgggaccctgagatggggggaaagccgagaaggaagaaccctcaggaaggcctgtacaatgaactgcagaaagataagatggcggaggcctacagtgagattgggatgaaaggcgagcgccggaggggcaaggggcacgatggcctttaccagggtctcagtacagccaccaaggacacctacgacgcccttcacatgcaggccctgccccctcgctaa

SEQ ID NO: 26 - protein, 749 aa, synthetic construct
MALPVTALLLPLALLLHAARPEIVLTQSPATLSLSPGERATLSCRASQSVSSYLAWYQQKPGQAPRLLIYDASNRATGIPARFSGSGSGTDFTLTISSLEPEDFAVYYCQQRSNWPITFGQGTRLEIKGSTSGGGSGGGSGGGGSSEVQLVESGGGLVQPGRSLRLSCAASGFTFNDYAMHWVRQAPGKGLEWVSTISWNSGSIGYADSVKGRFTISRDNAKKSLYLQMNSLRAEDTALYYCAKDIQYGNYYYGMDVWGQGTTVTVSSGGGGSDIQMTQSPSSLSASVGDRVTITCRASQGISNYLNWYQQKPGKAPKPLIYYTSNLQSGVPSRFSGSGSGTDYTLTISSLQPEDFATYYCMGQTISSYTFGQGTKLEIKGGGGSGGGGSGGGGSEVQLVESGGGLVQPGGSLRLSCAASGFTFSNFDMAWVRQAPGKGLVWVSSITTGADHAIYADSVKGRFTISRDNAKNTLYLQMNSLRAEDTAVYYCVRHGYYDGYHLFDYWGQGTLVTVSSFVPVFLPAKPTTTPAPRPPTPAPTIASQPLSLRPEACRPAAGGAVHTRGLDFACDIYIWAPLAGTCGVLLLSLVITLYCKRGRKKLLYIFKQPFMRPVQTTQEEDGCSCRFPEEEEGGCELRVKFSRSADAPAYQQGQNQLYNELNLGRREEYDVLDKRRGRDPEMGGKPRRKNPQEGLYNELQKDKMAEAYSEIGMKGERRRGKGHDGLYQGLSTATKDTYDALHMQALPPR

SEQ ID NO: 27 - DNA, 63 bp, synthetic construct; identical to SEQ ID NO: 1
  source 1..63: mol_type = other DNA

SEQ ID NO: 28 - DNA, 366 bp, synthetic construct; identical to SEQ ID NO: 7
  source 1..366: mol_type = other DNA

SEQ ID NO: 29 - DNA, 54 bp, synthetic construct; identical to SEQ ID NO: 5
  source 1..54: mol_type = other DNA

SEQ ID NO: 30 - DNA, 321 bp, synthetic construct; identical to SEQ ID NO: 3
  source 1..321: mol_type = other DNA

SEQ ID NO: 31 - DNA, 15 bp, synthetic construct
  source 1..15: mol_type = other DNA
ggaggtggtggatcc

SEQ ID NO: 32 - DNA, 321 bp, synthetic construct; identical to SEQ ID NO: 11
  source 1..321: mol_type = other DNA

SEQ ID NO: 33 - DNA, 45 bp, synthetic construct; identical to SEQ ID NO: 13
  source 1..45: mol_type = other DNA

SEQ ID NO: 34 - DNA, 363 bp, synthetic construct; identical to SEQ ID NO: 15
  source 1..363: mol_type = other DNA

SEQ ID NO: 35 - DNA, 165 bp, synthetic construct; identical to SEQ ID NO: 17
  source 1..165: mol_type = other DNA

SEQ ID NO: 36 - DNA, 72 bp, synthetic construct; identical to SEQ ID NO: 19
  source 1..72: mol_type = other DNA

SEQ ID NO: 37 - DNA, 126 bp, synthetic construct; identical to SEQ ID NO: 21
  source 1..126: mol_type = other DNA

SEQ ID NO: 38 - DNA, 339 bp, synthetic construct; identical to SEQ ID NO: 23
  source 1..339: mol_type = other DNA

SEQ ID NO: 39 - DNA, 2250 bp, synthetic construct
  source 1..2250: mol_type = other DNA
atggccttaccagtgaccgccttgctcctgccgctggccttgctgctccacgccgccaggccggaagtgcagctggtggagtctgggggaggcttggtacagcctggcaggtccctgagactctcctgtgcagcctctggattcacctttaatgattatgccatgcactgggtccggcaagctccagggaagggcctggagtgggtctcaactattagttggaatagtggttccataggctatgcggactctgtgaagggccgattcaccatctccagagacaacgccaagaagtccctgtatctgcaaatgaacagtctgagagctgaggacacggccttgtattactgtgcaaaagatatacagtacggcaactactactacggtatggacgtctggggccaagggaccacggtcaccgtctcctcaggcagtactagcggtggtggctccgggggcggttccggtgggggcggcagcagcgaaattgtgttgacacagtctccagccaccctgtctttgtctccaggggaaagagccaccctctcctgcagggccagtcagagtgttagcagctacttagcctggtaccaacagaaacctggccaggctcccaggctcctcatctatgatgcatccaacagggccactggcatcccagccaggttcagtggcagtgggtctgggacagacttcactctcaccatcagcagcctagagcctgaagattttgcagtttattactgtcagcagcgtagcaactggccgatcaccttcggccaagggacacgactggagattaaaggaggtggtggatccgacatccagatgacccagtccccctcctccctgtccgcctccgtgggcgaccgggtgaccatcacctgccgggcctcccagggcatctccaactacctgaactggtaccagcagaagcccggcaaggcccccaagcccctgatctactacacctccaacctgcagtccggcgtgccctcccggttctccggctccggctccggcaccgactacaccctgaccatctcctccctgcagcccgaggacttcgccacctactactgcatgggccagaccatctcctcctacaccttcggccagggcaccaagctggagatcaagggtggcggtggctcgggcggtggtgggtcgggtggcggcggatctgaggtgcagctggtggagtccggcggcggcctggtgcagcccggcggctccctgcggctgtcctgcgccgcctccggcttcaccttctccaacttcgacatggcctgggtgcggcaggcccccggcaagggcctggtgtgggtgtcctccatcaccaccggcgccgaccacgccatctacgccgactccgtgaagggccggttcaccatctcccgggacaacgccaagaacaccctgtacctgcagatgaactccctgcgggccgaggacaccgccgtgtactactgcgtgcggcacggctactacgacggctaccacctgttcgactactggggccagggcaccctggtgaccgtgtcctccttcgtgccggtcttcctgccagcgaagcccaccacgacgccagcgccgcgaccaccaacaccggcgcccaccatcgcgtcgcagcccctgtccctgcgcccagaggcgtgccggccagcggcggggggcgcagtgcacacgagggggctggacttcgcctgtgatatctacatctgggcgcccttggccgggacttgtggggtccttctcctgtcactggttatcaccctttactgcaaacggggcagaaagaaactcctgtatatattcaaacaaccatttatgagaccagtacaaactactcaagaggaagatggctgtagctgccgatttccagaagaagaagaaggaggatgtgaactgagagtgaagttcagcaggagcgcagacgcccccgcgtaccagcagggccagaaccagctctataacgagctcaatctaggacgaagagaggagtacgatgttttggacaagagacgtggccgggaccctgagatggggggaaagccgagaaggaagaaccctcaggaaggcctgtacaatgaactgcagaaagataagatggcggaggcctacagtgagattgggatgaaaggcgagcgccggaggggcaaggggcacgatggcctttaccagggtctcagtacagccaccaaggacacctacgacgcccttcacatgcaggccctgccccctcgctaa

SEQ ID NO: 40 - protein, 749 aa, synthetic construct
MALPVTALLLPLALLLHAARPEVQLVESGGGLVQPGRSLRLSCAASGFTFNDYAMHWVRQAPGKGLEWVSTISWNSGSIGYADSVKGRFTISRDNAKKSLYLQMNSLRAEDTALYYCAKDIQYGNYYYGMDVWGQGTTVTVSSGSTSGGGSGGGSGGGGSSEIVLTQSPATLSLSPGERATLSCRASQSVSSYLAWYQQKPGQAPRLLIYDASNRATGIPARFSGSGSGTDFTLTISSLEPEDFAVYYCQQRSNWPITFGQGTRLEIKGGGGSDIQMTQSPSSLSASVGDRVTITCRASQGISNYLNWYQQKPGKAPKPLIYYTSNLQSGVPSRFSGSGSGTDYTLTISSLQPEDFATYYCMGQTISSYTFGQGTKLEIKGGGGSGGGGSGGGGSEVQLVESGGGLVQPGGSLRLSCAASGFTFSNFDMAWVRQAPGKGLVWVSSITTGADHAIYADSVKGRFTISRDNAKNTLYLQMNSLRAEDTAVYYCVRHGYYDGYHLFDYWGQGTLVTVSSFVPVFLPAKPTTTPAPRPPTPAPTIASQPLSLRPEACRPAAGGAVHTRGLDFACDIYIWAPLAGTCGVLLLSLVITLYCKRGRKKLLYIFKQPFMRPVQTTQEEDGCSCRFPEEEEGGCELRVKFSRSADAPAYQQGQNQLYNELNLGRREEYDVLDKRRGRDPEMGGKPRRKNPQEGLYNELQKDKMAEAYSEIGMKGERRRGKGHDGLYQGLSTATKDTYDALHMQALPPR

SEQ ID NO: 41 - DNA, 63 bp, synthetic construct; identical to SEQ ID NO: 1
  source 1..63: mol_type = other DNA

SEQ ID NO: 42 - DNA, 366 bp, synthetic construct; identical to SEQ ID NO: 7
  source 1..366: mol_type = other DNA

SEQ ID NO: 43 - DNA, 54 bp, synthetic construct; identical to SEQ ID NO: 5
  source 1..54: mol_type = other DNA

SEQ ID NO: 44 - DNA, 321 bp, synthetic construct; identical to SEQ ID NO: 3
  source 1..321: mol_type = other DNA

SEQ ID NO: 45 - DNA, 15 bp, synthetic construct
  source 1..15: mol_type = other DNA
ggaggtggtggatcc

SEQ ID NO: 46 - DNA, 363 bp, synthetic construct; identical to SEQ ID NO: 15
  source 1..363: mol_type = other DNA

SEQ ID NO: 47 - DNA, 45 bp, synthetic construct; identical to SEQ ID NO: 13
  source 1..45: mol_type = other DNA

SEQ ID NO: 48 - DNA, 321 bp, synthetic construct; identical to SEQ ID NO: 11
  source 1..321: mol_type = other DNA

SEQ ID NO: 49 - DNA, 165 bp, synthetic construct; identical to SEQ ID NO: 17
  source 1..165: mol_type = other DNA

SEQ ID NO: 50 - DNA, 72 bp, synthetic construct; identical to SEQ ID NO: 19
  source 1..72: mol_type = other DNA

SEQ ID NO: 51 - DNA, 126 bp, synthetic construct; identical to SEQ ID NO: 21
  source 1..126: mol_type = other DNA

SEQ ID NO: 52 - DNA, 339 bp, synthetic construct; identical to SEQ ID NO: 23
  source 1..339: mol_type = other DNA

SEQ ID NO: 53 - DNA, 2250 bp, synthetic construct
  source 1..2250: mol_type = other DNA
atggccttaccagtgaccgccttgctcctgccgctggccttgctgctccacgccgccaggccggaagtgcagctggtggagtctgggggaggcttggtacagcctggcaggtccctgagactctcctgtgcagcctctggattcacctttaatgattatgccatgcactgggtccggcaagctccagggaagggcctggagtgggtctcaactattagttggaatagtggttccataggctatgcggactctgtgaagggccgattcaccatctccagagacaacgccaagaagtccctgtatctgcaaatgaacagtctgagagctgaggacacggccttgtattactgtgcaaaagatatacagtacggcaactactactacggtatggacgtctggggccaagggaccacggtcaccgtctcctcaggcagtactagcggtggtggctccgggggcggttccggtgggggcggcagcagcgaaattgtgttgacacagtctccagccaccctgtctttgtctccaggggaaagagccaccctctcctgcagggccagtcagagtgttagcagctacttagcctggtaccaacagaaacctggccaggctcccaggctcctcatctatgatgcatccaacagggccactggcatcccagccaggttcagtggcagtgggtctgggacagacttcactctcaccatcagcagcctagagcctgaagattttgcagtttattactgtcagcagcgtagcaactggccgatcaccttcggccaagggacacgactggagattaaaggaggtggtggatccgaggtgcagctggtggagtccggcggcggcctggtgcagcccggcggctccctgcggctgtcctgcgccgcctccggcttcaccttctccaacttcgacatggcctgggtgcggcaggcccccggcaagggcctggtgtgggtgtcctccatcaccaccggcgccgaccacgccatctacgccgactccgtgaagggccggttcaccatctcccgggacaacgccaagaacaccctgtacctgcagatgaactccctgcgggccgaggacaccgccgtgtactactgcgtgcggcacggctactacgacggctaccacctgttcgactactggggccagggcaccctggtgaccgtgtcctccggtggcggtggctcgggcggtggtgggtcgggtggcggcggatctgacatccagatgacccagtccccctcctccctgtccgcctccgtgggcgaccgggtgaccatcacctgccgggcctcccagggcatctccaactacctgaactggtaccagcagaagcccggcaaggcccccaagcccctgatctactacacctccaacctgcagtccggcgtgccctcccggttctccggctccggctccggcaccgactacaccctgaccatctcctccctgcagcccgaggacttcgccacctactactgcatgggccagaccatctcctcctacaccttcggccagggcaccaagctggagatcaagttcgtgccggtcttcctgccagcgaagcccaccacgacgccagcgccgcgaccaccaacaccggcgcccaccatcgcgtcgcagcccctgtccctgcgcccagaggcgtgccggccagcggcggggggcgcagtgcacacgagggggctggacttcgcctgtgatatctacatctgggcgcccttggccgggacttgtggggtccttctcctgtcactggttatcaccctttactgcaaacggggcagaaagaaactcctgtatatattcaaacaaccatttatgagaccagtacaaactactcaagaggaagatggctgtagctgccgatttccagaagaagaagaaggaggatgtgaactgagagtgaagttcagcaggagcgcagacgcccccgcgtaccagcagggccagaaccagctctataacgagctcaatctaggacgaagagaggagtacgatgttttggacaagagacgtggccgggaccctgagatggggggaaagccgagaaggaagaaccctcaggaaggcctgtacaatgaactgcagaaagataagatggcggaggcctacagtgagattgggatgaaaggcgagcgccggaggggcaaggggcacgatggcctttaccagggtctcagtacagccaccaaggacacctacgacgcccttcacatgcaggccctgccccctcgctaa

SEQ ID NO: 54 - protein, 749 aa, synthetic construct
MALPVTALLLPLALLLHAARPEVQLVESGGGLVQPGRSLRLSCAASGFTFNDYAMHWVRQAPGKGLEWVSTISWNSGSIGYADSVKGRFTISRDNAKKSLYLQMNSLRAEDTALYYCAKDIQYGNYYYGMDVWGQGTTVTVSSGSTSGGGSGGGSGGGGSSEIVLTQSPATLSLSPGERATLSCRASQSVSSYLAWYQQKPGQAPRLLIYDASNRATGIPARFSGSGSGTDFTLTISSLEPEDFAVYYCQQRSNWPITFGQGTRLEIKGGGGSEVQLVESGGGLVQPGGSLRLSCAASGFTFSNFDMAWVRQAPGKGLVWVSSITTGADHAIYADSVKGRFTISRDNAKNTLYLQMNSLRAEDTAVYYCVRHGYYDGYHLFDYWGQGTLVTVSSGGGGSGGGGSGGGGSDIQMTQSPSSLSASVGDRVTITCRASQGISNYLNWYQQKPGKAPKPLIYYTSNLQSGVPSRFSGSGSGTDYTLTISSLQPEDFATYYCMGQTISSYTFGQGTKLEIKFVPVFLPAKPTTTPAPRPPTPAPTIASQPLSLRPEACRPAAGGAVHTRGLDFACDIYIWAPLAGTCGVLLLSLVITLYCKRGRKKLLYIFKQPFMRPVQTTQEEDGCSCRFPEEEEGGCELRVKFSRSADAPAYQQGQNQLYNELNLGRREEYDVLDKRRGRDPEMGGKPRRKNPQEGLYNELQKDKMAEAYSEIGMKGERRRGKGHDGLYQGLSTATKDTYDALHMQALPPR

SEQ ID NO: 55 - DNA, 63 bp, synthetic construct; identical to SEQ ID NO: 1
  source 1..63: mol_type = other DNA

SEQ ID NO: 56 - DNA, 321 bp, synthetic construct; identical to SEQ ID NO: 3
  source 1..321: mol_type = other DNA

SEQ ID NO: 57 - DNA, 54 bp, synthetic construct; identical to SEQ ID NO: 5
  source 1..54: mol_type = other DNA

SEQ ID NO: 58 - DNA, 366 bp, synthetic construct; identical to SEQ ID NO: 7
  source 1..366: mol_type = other DNA

SEQ ID NO: 59 - DNA, 15 bp, synthetic construct
  source 1..15: mol_type = other DNA
ggaggtggtggatcc

SEQ ID NO: 60 - DNA, 363 bp, synthetic construct; identical to SEQ ID NO: 15
  source 1..363: mol_type = other DNA

SEQ ID NO: 61 - DNA, 45 bp, synthetic construct; identical to SEQ ID NO: 13
  source 1..45: mol_type = other DNA

SEQ ID NO: 62 - DNA, 321 bp, synthetic construct; identical to SEQ ID NO: 11
  source 1..321: mol_type = other DNA

SEQ ID NO: 63 - DNA, 165 bp, synthetic construct; identical to SEQ ID NO: 17
  source 1..165: mol_type = other DNA

SEQ ID NO: 64 - DNA, 72 bp, synthetic construct; identical to SEQ ID NO: 19
  source 1..72: mol_type = other DNA

SEQ ID NO: 65 - DNA, 126 bp, synthetic construct; identical to SEQ ID NO: 21
  source 1..126: mol_type = other DNA

SEQ ID NO: 66 - DNA, 339 bp, synthetic construct; identical to SEQ ID NO: 23
  source 1..339: mol_type = other DNA

SEQ ID NO: 67 - DNA, 2250 bp, synthetic construct
  source 1..2250: mol_type = other DNA
atggccttaccagtgaccgccttgctcctgccgctggccttgctgctccacgccgccaggccggaaattgtgttgacacagtctccagccaccctgtctttgtctccaggggaaagagccaccctctcctgcagggccagtcagagtgttagcagctacttagcctggtaccaacagaaacctggccaggctcccaggctcctcatctatgatgcatccaacagggccactggcatcccagccaggttcagtggcagtgggtctgggacagacttcactctcaccatcagcagcctagagcctgaagattttgcagtttattactgtcagcagcgtagcaactggccgatcaccttcggccaagggacacgactggagattaaaggcagtactagcggtggtggctccgggggcggttccggtgggggcggcagcagcgaagtgcagctggtggagtctgggggaggcttggtacagcctggcaggtccctgagactctcctgtgcagcctctggattcacctttaatgattatgccatgcactgggtccggcaagctccagggaagggcctggagtgggtctcaactattagttggaatagtggttccataggctatgcggactctgtgaagggccgattcaccatctccagagacaacgccaagaagtccctgtatctgcaaatgaacagtctgagagctgaggacacggccttgtattactgtgcaaaagatatacagtacggcaactactactacggtatggacgtctggggccaagggaccacggtcaccgtctcctcaggaggtggtggatccgaggtgcagctggtggagtccggcggcggcctggtgcagcccggcggctccctgcggctgtcctgcgccgcctccggcttcaccttctccaacttcgacatggcctgggtgcggcaggcccccggcaagggcctggtgtgggtgtcctccatcaccaccggcgccgaccacgccatctacgccgactccgtgaagggccggttcaccatctcccgggacaacgccaagaacaccctgtacctgcagatgaactccctgcgggccgaggacaccgccgtgtactactgcgtgcggcacggctactacgacggctaccacctgttcgactactggggccagggcaccctggtgaccgtgtcctccggtggcggtggctcgggcggtggtgggtcgggtggcggcggatctgacatccagatgacccagtccccctcctccctgtccgcctccgtgggcgaccgggtgaccatcacctgccgggcctcccagggcatctccaactacctgaactggtaccagcagaagcccggcaaggcccccaagcccctgatctactacacctccaacctgcagtccggcgtgccctcccggttctccggctccggctccggcaccgactacaccctgaccatctcctccctgcagcccgaggacttcgccacctactactgcatgggccagaccatctcctcctacaccttcggccagggcaccaagctggagatcaagttcgtgccggtcttcctgccagcgaagcccaccacgacgccagcgccgcgaccaccaacaccggcgcccaccatcgcgtcgcagcccctgtccctgcgcccagaggcgtgccggccagcggcggggggcgcagtgcacacgagggggctggacttcgcctgtgatatctacatctgggcgcccttggccgggacttgtggggtccttctcctgtcactggttatcaccctttactgcaaacggggcagaaagaaactcctgtatatattcaaacaaccatttatgagaccagtacaaactactcaagaggaagatggctgtagctgccgatttccagaagaagaagaaggaggatgtgaactgagagtgaagttcagcaggagcgcagacgcccccgcgtaccagcagggccagaaccagctctataacgagctcaatctaggacgaagagaggagtacgatgttttggacaagagacgtggccgggaccctgagatggggggaaagccgagaaggaagaaccctcaggaaggcctgtacaatgaactgcagaaagataagatggcggaggcctacagtgagattgggatgaaaggcgagcgccggaggggcaaggggcacgatggcctttaccagggtctcagtacagccaccaaggacacctacgacgcccttcacatgcaggccctgccccctcgctaa

SEQ ID NO: 68 - protein, 749 aa, synthetic construct
MALPVTALLLPLALLLHAARPEIVLTQSPATLSLSPGERATLSCRASQSVSSYLAWYQQKPGQAPRLLIYDASNRATGIPARFSGSGSGTDFTLTISSLEPEDFAVYYCQQRSNWPITFGQGTRLEIKGSTSGGGSGGGSGGGGSSEVQLVESGGGLVQPGRSLRLSCAASGFTFNDYAMHWVRQAPGKGLEWVSTISWNSGSIGYADSVKGRFTISRDNAKKSLYLQMNSLRAEDTALYYCAKDIQYGNYYYGMDVWGQGTTVTVSSGGGGSEVQLVESGGGLVQPGGSLRLSCAASGFTFSNFDMAWVRQAPGKGLVWVSSITTGADHAIYADSVKGRFTISRDNAKNTLYLQMNSLRAEDTAVYYCVRHGYYDGYHLFDYWGQGTLVTVSSGGGGSGGGGSGGGGSDIQMTQSPSSLSASVGDRVTITCRASQGISNYLNWYQQKPGKAPKPLIYYTSNLQSGVPSRFSGSGSGTDYTLTISSLQPEDFATYYCMGQTISSYTFGQGTKLEIKFVPVFLPAKPTTTPAPRPPTPAPTIASQPLSLRPEACRPAAGGAVHTRGLDFACDIYIWAPLAGTCGVLLLSLVITLYCKRGRKKLLYIFKQPFMRPVQTTQEEDGCSCRFPEEEEGGCELRVKFSRSADAPAYQQGQNQLYNELNLGRREEYDVLDKRRGRDPEMGGKPRRKNPQEGLYNELQKDKMAEAYSEIGMKGERRRGKGHDGLYQGLSTATKDTYDALHMQALPPR

SEQ ID NO: 69 - DNA, 63 bp, synthetic construct; identical to SEQ ID NO: 1
  source 1..63: mol_type = other DNA

SEQ ID NO: 70 - DNA, 321 bp, synthetic construct; identical to SEQ ID NO: 3
  source 1..321: mol_type = other DNA

SEQ ID NO: 71 - DNA, 54 bp, synthetic construct; identical to SEQ ID NO: 5
  source 1..54: mol_type = other DNA

SEQ ID NO: 72 - DNA, 366 bp, synthetic construct; identical to SEQ ID NO: 7
  source 1..366: mol_type = other DNA

SEQ ID NO: 73 - DNA, 15 bp, synthetic construct
  source 1..15: mol_type = other DNA
ggaggtggtggatcc

SEQ ID NO: 74 - DNA, 363 bp, synthetic construct; identical to SEQ ID NO: 15
  source 1..363: mol_type = other DNA

SEQ ID NO: 75 - DNA, 45 bp, synthetic construct; identical to SEQ ID NO: 13
  source 1..45: mol_type = other DNA

SEQ ID NO: 76 - DNA, 321 bp, synthetic construct; identical to SEQ ID NO: 11
  source 1..321: mol_type = other DNA

SEQ ID NO: 77 - DNA, 36 bp, synthetic construct
  source 1..36: mol_type = other DNA
gagagcaagtacggaccgccctgccccccttgccct

SEQ ID NO: 78 - protein, 12 aa, synthetic construct
ESKYGPPCPPCP

SEQ ID NO: 79 - DNA, 84 bp, synthetic construct
  source 1..84: mol_type = other DNA
atgttctgggtgctggtggtggtcggaggcgtgctggcctgctacagcctgctggtcaccgtggccttcatcatcttttgggtg

SEQ ID NO: 80 - protein, 28 aa, synthetic construct
MFWVLVVVGGVLACYSLLVTVAFIIFWV

SEQ ID NO: 81 - DNA, 126 bp, synthetic construct; identical to SEQ ID NO: 21
  source 1..126: mol_type = other DNA

SEQ ID NO: 82 - DNA, 336 bp, synthetic construct
  source 1..336: mol_type = other DNA
cgggtgaagttcagcagaagcgccgacgcccctgcctaccagcagggccagaatcagctgtacaacgagctgaacctgggcagaagggaagagtacgacgtcctggataagcggagaggccgggaccctgagatgggcggcaagcctcggcggaagaacccccaggaaggcctgtataacgaactgcagaaagacaagatggccgaggcctacagcgagatcggcatgaagggcgagcggaggcggggcaagggccacgacggcctgtatcagggcctgtccaccgccaccaaggatacctacgacgccctgcacatgcaggccctgcccccaagg

SEQ ID NO: 83 - DNA, 2133 bp, synthetic construct
  source 1..2133: mol_type = other DNA
atggccttaccagtgaccgccttgctcctgccgctggccttgctgctccacgccgccaggccggaaattgtgttgacacagtctccagccaccctgtctttgtctccaggggaaagagccaccctctcctgcagggccagtcagagtgttagcagctacttagcctggtaccaacagaaacctggccaggctcccaggctcctcatctatgatgcatccaacagggccactggcatcccagccaggttcagtggcagtgggtctgggacagacttcactctcaccatcagcagcctagagcctgaagattttgcagtttattactgtcagcagcgtagcaactggccgatcaccttcggccaagggacacgactggagattaaaggcagtactagcggtggtggctccgggggcggttccggtgggggcggcagcagcgaagtgcagctggtggagtctgggggaggcttggtacagcctggcaggtccctgagactctcctgtgcagcctctggattcacctttaatgattatgccatgcactgggtccggcaagctccagggaagggcctggagtgggtctcaactattagttggaatagtggttccataggctatgcggactctgtgaagggccgattcaccatctccagagacaacgccaagaagtccctgtatctgcaaatgaacagtctgagagctgaggacacggccttgtattactgtgcaaaagatatacagtacggcaactactactacggtatggacgtctggggccaagggaccacggtcaccgtctcctcaggaggtggtggatccgaggtgcagctggtggagtccggcggcggcctggtgcagcccggcggctccctgcggctgtcctgcgccgcctccggcttcaccttctccaacttcgacatggcctgggtgcggcaggcccccggcaagggcctggtgtgggtgtcctccatcaccaccggcgccgaccacgccatctacgccgactccgtgaagggccggttcaccatctcccgggacaacgccaagaacaccctgtacctgcagatgaactccctgcgggccgaggacaccgccgtgtactactgcgtgcggcacggctactacgacggctaccacctgttcgactactggggccagggcaccctggtgaccgtgtcctccggtggcggtggctcgggcggtggtgggtcgggtggcggcggatctgacatccagatgacccagtccccctcctccctgtccgcctccgtgggcgaccgggtgaccatcacctgccgggcctcccagggcatctccaactacctgaactggtaccagcagaagcccggcaaggcccccaagcccctgatctactacacctccaacctgcagtccggcgtgccctcccggttctccggctccggctccggcaccgactacaccctgaccatctcctccctgcagcccgaggacttcgccacctactactgcatgggccagaccatctcctcctacaccttcggccagggcaccaagctggagatcaaggagagcaagtacggaccgccctgccccccttgccctatgttctgggtgctggtggtggtcggaggcgtgctggcctgctacagcctgctggtcaccgtggccttcatcatcttttgggtgaaacggggcagaaagaaactcctgtatatattcaaacaaccatttatgagaccagtacaaactactcaagaggaagatggctgtagctgccgatttccagaagaagaagaaggaggatgtgaactgcgggtgaagttcagcagaagcgccgacgcccctgcctaccagcagggccagaatcagctgtacaacgagctgaacctgggcagaagggaagagtacgacgtcctggataagcggagaggccgggaccctgagatgggcggcaagcctcggcggaagaacccccaggaaggcctgtataacgaactgcagaaagacaagatggccgaggcctacagcgagatcggcatgaagggcgagcggaggcggggcaagggccacgacggcctgtatcagggcctgtccaccgccaccaaggatacctacgacgccctgcacatgcaggccctgcccccaaggtaa

SEQ ID NO: 84 - protein, 710 aa, synthetic construct
MALPVTALLLPLALLLHAARPEIVLTQSPATLSLSPGERATLSCRASQSVSSYLAWYQQKPGQAPRLLIYDASNRATGIPARFSGSGSGTDFTLTISSLEPEDFAVYYCQQRSNWPITFGQGTRLEIKGSTSGGGSGGGSGGGGSSEVQLVESGGGLVQPGRSLRLSCAASGFTFNDYAMHWVRQAPGKGLEWVSTISWNSGSIGYADSVKGRFTISRDNAKKSLYLQMNSLRAEDTALYYCAKDIQYGNYYYGMDVWGQGTTVTVSSGGGGSEVQLVESGGGLVQPGGSLRLSCAASGFTFSNFDMAWVRQAPGKGLVWVSSITTGADHAIYADSVKGRFTISRDNAKNTLYLQMNSLRAEDTAVYYCVRHGYYDGYHLFDYWGQGTLVTVSSGGGGSGGGGSGGGGSDIQMTQSPSSLSASVGDRVTITCRASQGISNYLNWYQQKPGKAPKPLIYYTSNLQSGVPSRFSGSGSGTDYTLTISSLQPEDFATYYCMGQTISSYTFGQGTKLEIKESKYGPPCPPCPMFWVLVVVGGVLACYSLLVTVAFIIFWVKRGRKKLLYIFKQPFMRPVQTTQEEDGCSCRFPEEEEGGCELRVKFSRSADAPAYQQGQNQLYNELNLGRREEYDVLDKRRGRDPEMGGKPRRKNPQEGLYNELQKDKMAEAYSEIGMKGERRRGKGHDGLYQGLSTATKDTYDALHMQALPPR

SEQ ID NO: 85 - DNA, 63 bp, synthetic construct; identical to SEQ ID NO: 1
  source 1..63: mol_type = other DNA

SEQ ID NO: 86 - DNA, 321 bp, synthetic construct; identical to SEQ ID NO: 3
  source 1..321: mol_type = other DNA

SEQ ID NO: 87 - DNA, 54 bp, synthetic construct; identical to SEQ ID NO: 5
  source 1..54: mol_type = other DNA

SEQ ID NO: 88 - DNA, 366 bp, synthetic construct; identical to SEQ ID NO: 7
  source 1..366: mol_type = other DNA

SEQ ID NO: 89 - DNA, 15 bp, synthetic construct
  source 1..15: mol_type = other DNA
ggaggtggtggatcc

SEQ ID NO: 90 - DNA, 321 bp, synthetic construct; identical to SEQ ID NO: 11
  source 1..321: mol_type = other DNA

SEQ ID NO: 91 - DNA, 45 bp, synthetic construct; identical to SEQ ID NO: 13
  source 1..45: mol_type = other DNA

SEQ ID NO: 92 - DNA, 363 bp, synthetic construct; identical to SEQ ID NO: 15
  source 1..363: mol_type = other DNA

SEQ ID NO: 93 - DNA, 36 bp, synthetic construct; identical to SEQ ID NO: 77
  source 1..36: mol_type = other DNA

SEQ ID NO: 94 - DNA, 84 bp, synthetic construct; identical to SEQ ID NO: 79
  source 1..84: mol_type = other DNA

SEQ ID NO: 95 - DNA, 126 bp, synthetic construct; identical to SEQ ID NO: 21
  source 1..126: mol_type = other DNA

SEQ ID NO: 96 - DNA, 336 bp, synthetic construct; identical to SEQ ID NO: 82
  source 1..336: mol_type = other DNA

SEQ ID NO: 97 - DNA, 2133 bp, synthetic construct
  source 1..2133: mol_type = other DNA
atggccttaccagtgaccgccttgctcctgccgctggccttgctgctccacgccgccaggccggaaattgtgttgacacagtctccagccaccctgtctttgtctccaggggaaagagccaccctctcctgcagggccagtcagagtgttagcagctacttagcctggtaccaacagaaacctggccaggctcccaggctcctcatctatgatgcatccaacagggccactggcatcccagccaggttcagtggcagtgggtctgggacagacttcactctcaccatcagcagcctagagcctgaagattttgcagtttattactgtcagcagcgtagcaactggccgatcaccttcggccaagggacacgactggagattaaaggcagtactagcggtggtggctccgggggcggttccggtgggggcggcagcagcgaagtgcagctggtggagtctgggggaggcttggtacagcctggcaggtccctgagactctcctgtgcagcctctggattcacctttaatgattatgccatgcactgggtccggcaagctccagggaagggcctggagtgggtctcaactattagttggaatagtggttccataggctatgcggactctgtgaagggccgattcaccatctccagagacaacgccaagaagtccctgtatctgcaaatgaacagtctgagagctgaggacacggccttgtattactgtgcaaaagatatacagtacggcaactactactacggtatggacgtctggggccaagggaccacggtcaccgtctcctcaggaggtggtggatccgacatccagatgacccagtccccctcctccctgtccgcctccgtgggcgaccgggtgaccatcacctgccgggcctcccagggcatctccaactacctgaactggtaccagcagaagcccggcaaggcccccaagcccctgatctactacacctccaacctgcagtccggcgtgccctcccggttctccggctccggctccggcaccgactacaccctgaccatctcctccctgcagcccgaggacttcgccacctactactgcatgggccagaccatctcctcctacaccttcggccagggcaccaagctggagatcaagggtggcggtggctcgggcggtggtgggtcgggtggcggcggatctgaggtgcagctggtggagtccggcggcggcctggtgcagcccggcggctccctgcggctgtcctgcgccgcctccggcttcaccttctccaacttcgacatggcctgggtgcggcaggcccccggcaagggcctggtgtgggtgtcctccatcaccaccggcgccgaccacgccatctacgccgactccgtgaagggccggttcaccatctcccgggacaacgccaagaacaccctgtacctgcagatgaactccctgcgggccgaggacaccgccgtgtactactgcgtgcggcacggctactacgacggctaccacctgttcgactactggggccagggcaccctggtgaccgtgtcctccgagagcaagtacggaccgccctgccccccttgccctatgttctgggtgctggtggtggtcggaggcgtgctggcctgctacagcctgctggtcaccgtggccttcatcatcttttgggtgaaacggggcagaaagaaactcctgtatatattcaaacaaccatttatgagaccagtacaaactactcaagaggaagatggctgtagctgccgatttccagaagaagaagaaggaggatgtgaactgcgggtgaagttcagcagaagcgccgacgcccctgcctaccagcagggccagaatcagctgtacaacgagctgaacctgggcagaagggaagagtacgacgtcctggataagcggagaggccgggaccctgagatgggcggcaagcctcggcggaagaacccccaggaaggcctgtataacgaactgcagaaagacaagatggccgaggcctacagcgagatcggcatgaagggcgagcggaggcggggcaagggccacgacggcctgtatcagggcctgtccaccgccaccaaggatacctacgacgccctgcacatgcaggccctgcccccaaggtaa

SEQ ID NO: 98 - protein, 710 aa, synthetic construct
MALPVTALLLPLALLLHAARPEIVLTQSPATLSLSPGERATLSCRASQSVSSYLAWYQQKPGQAPRLLIYDASNRATGIPARFSGSGSGTDFTLTISSLEPEDFAVYYCQQRSNWPITFGQGTRLEIKGSTSGGGSGGGSGGGGSSEVQLVESGGGLVQPGRSLRLSCAASGFTFNDYAMHWVRQAPGKGLEWVSTISWNSGSIGYADSVKGRFTISRDNAKKSLYLQMNSLRAEDTALYYCAKDIQYGNYYYGMDVWGQGTTVTVSSGGGGSDIQMTQSPSSLSASVGDRVTITCRASQGISNYLNWYQQKPGKAPKPLIYYTSNLQSGVPSRFSGSGSGTDYTLTISSLQPEDFATYYCMGQTISSYTFGQGTKLEIKGGGGSGGGGSGGGGSEVQLVESGGGLVQPGGSLRLSCAASGFTFSNFDMAWVRQAPGKGLVWVSSITTGADHAIYADSVKGRFTISRDNAKNTLYLQMNSLRAEDTAVYYCVRHGYYDGYHLFDYWGQGTLVTVSSESKYGPPCPPCPMFWVLVVVGGVLACYSLLVTVAFIIFWVKRGRKKLLYIFKQPFMRPVQTTQEEDGCSCRFPEEEEGGCELRVKFSRSADAPAYQQGQNQLYNELNLGRREEYDVLDKRRGRDPEMGGKPRRKNPQEGLYNELQKDKMAEAYSEIGMKGERRRGKGHDGLYQGLSTATKDTYDALHMQALPPR

SEQ ID NO: 99 - DNA, 63 bp, synthetic construct; identical to SEQ ID NO: 1
  source 1..63: mol_type = other DNA

SEQ ID NO: 100 - DNA, 366 bp, synthetic construct; identical to SEQ ID NO: 7
  source 1..366: mol_type = other DNA

SEQ ID NO: 101 - DNA, 54 bp, synthetic construct; identical to SEQ ID NO: 5
  source 1..54: mol_type = other DNA

SEQ ID NO: 102 - DNA, 321 bp, synthetic construct; identical to SEQ ID NO: 3
  source 1..321: mol_type = other DNA

SEQ ID NO: 103 - DNA, 15 bp, synthetic construct
  source 1..15: mol_type = other DNA
ggaggtggtggatcc

SEQ ID NO: 104 - DNA, 321 bp, synthetic construct; identical to SEQ ID NO: 11
  source 1..321: mol_type = other DNA

SEQ ID NO: 105 - DNA, 45 bp, synthetic construct; identical to SEQ ID NO: 13
  source 1..45: mol_type = other DNA

SEQ ID NO: 106 - DNA, 363 bp, synthetic construct; identical to SEQ ID NO: 15
  source 1..363: mol_type = other DNA

SEQ ID NO: 107 - DNA, 36 bp, synthetic construct; identical to SEQ ID NO: 77
  source 1..36: mol_type = other DNA

SEQ ID NO: 108 - DNA, 84 bp, synthetic construct; identical to SEQ ID NO: 79
  source 1..84: mol_type = other DNA

SEQ ID NO: 109 - DNA, 126 bp, synthetic construct; identical to SEQ ID NO: 21
  source 1..126: mol_type = other DNA

SEQ ID NO: 110 - DNA, 336 bp, synthetic construct; identical to SEQ ID NO: 82
  source 1..336: mol_type = other DNA

SEQ ID NO: 111 - DNA, 2133 bp, synthetic construct
  source 1..2133: mol_type = other DNA
atggccttaccagtgaccgccttgctcctgccgctggccttgctgctccacgccgccaggccggaagtgcagctggtggagtctgggggaggcttggtacagcctggcaggtccctgagactctcctgtgcagcctctggattcacctttaatgattatgccatgcactgggtccggcaagctccagggaagggcctggagtgggtctcaactattagttggaatagtggttccataggctatgcggactctgtgaagggccgattcaccatctccagagacaacgccaagaagtccctgtatctgcaaatgaacagtctgagagctgaggacacggccttgtattactgtgcaaaagatatacagtacggcaactactactacggtatggacgtctggggccaagggaccacggtcaccgtctcctcaggcagtactagcggtggtggctccgggggcggttccggtgggggcggcagcagcgaaattgtgttgacacagtctccagccaccctgtctttgtctccaggggaaagagccaccctctcctgcagggccagtcagagtgttagcagctacttagcctggtaccaacagaaacctggccaggctcccaggctcctcatctatgatgcatccaacagggccactggcatcccagccaggttcagtggcagtgggtctgggacagacttcactctcaccatcagcagcctagagcctgaagattttgcagtttattactgtcagcagcgtagcaactggccgatcaccttcggccaagggacacgactggagattaaaggaggtggtggatccgacatccagatgacccagtccccctcctccctgtccgcctccgtgggcgaccgggtgaccatcacctgccgggcctcccagggcatctccaactacctgaactggtaccagcagaagcccggcaaggcccccaagcccctgatctactacacctccaacctgcagtccggcgtgccctcccggttctccggctccggctccggcaccgactacaccctgaccatctcctccctgcagcccgaggacttcgccacctactactgcatgggccagaccatctcctcctacaccttcggccagggcaccaagctggagatcaagggtggcggtggctcgggcggtggtgggtcgggtggcggcggatctgaggtgcagctggtggagtccggcggcggcctggtgcagcccggcggctccctgcggctgtcctgcgccgcctccggcttcaccttctccaacttcgacatggcctgggtgcggcaggcccccggcaagggcctggtgtgggtgtcctccatcaccaccggcgccgaccacgccatctacgccgactccgtgaagggccggttcaccatctcccgggacaacgccaagaacaccctgtacctgcagatgaactccctgcgggccgaggacaccgccgtgtactactgcgtgcggcacggctactacgacggctaccacctgttcgactactggggccagggcaccctggtgaccgtgtcctccgagagcaagtacggaccgccctgccccccttgccctatgttctgggtgctggtggtggtcggaggcgtgctggcctgctacagcctgctggtcaccgtggccttcatcatcttttgggtgaaacggggcagaaagaaactcctgtatatattcaaacaaccatttatgagaccagtacaaactactcaagaggaagatggctgtagctgccgatttccagaagaagaagaaggaggatgtgaactgcgggtgaagttcagcagaagcgccgacgcccctgcctaccagcagggccagaatcagctgtacaacgagctgaacctgggcagaagggaagagtacgacgtcctggataagcggagaggccgggaccctgagatgggcggcaagcctcggcggaagaacccccaggaaggcctgtataacgaactgcagaaagacaagatggccgaggcctacagcgagatcggcatgaagggcgagcggaggcggggcaagggccacgacggcctgtatcagggcctgtccaccgccaccaaggatacctacgacgccctgcacatgcaggccctgcccccaaggtaa

SEQ ID NO: 112 - protein, 710 aa, synthetic construct
MALPVTALLLPLALLLHAARPEVQLVESGGGLVQPGRSLRLSCAASGFTFNDYAMHWVRQAPGKGLEWVSTISWNSGSIGYADSVKGRFTISRDNAKKSLYLQMNSLRAEDTALYYCAKDIQYGNYYYGMDVWGQGTTVTVSSGSTSGGGSGGGSGGGGSSEIVLTQSPATLSLSPGERATLSCRASQSVSSYLAWYQQKPGQAPRLLIYDASNRATGIPARFSGSGSGTDFTLTISSLEPEDFAVYYCQQRSNWPITFGQGTRLEIKGGGGSDIQMTQSPSSLSASVGDRVTITCRASQGISNYLNWYQQKPGKAPKPLIYYTSNLQSGVPSRFSGSGSGTDYTLTISSLQPEDFATYYCMGQTISSYTFGQGTKLEIKGGGGSGGGGSGGGGSEVQLVESGGGLVQPGGSLRLSCAASGFTFSNFDMAWVRQAPGKGLVWVSSITTGADHAIYADSVKGRFTISRDNAKNTLYLQMNSLRAEDTAVYYCVRHGYYDGYHLFDYWGQGTLVTVSSESKYGPPCPPCPMFWVLVVVGGVLACYSLLVTVAFIIFWVKRGRKKLLYIFKQPFMRPVQTTQEEDGCSCRFPEEEEGGCELRVKFSRSADAPAYQQGQNQLYNELNLGRREEYDVLDKRRGRDPEMGGKPRRKNPQEGLYNELQKDKMAEAYSEIGMKGERRRGKGHDGLYQGLSTATKDTYDALHMQALPPR

SEQ ID NO: 113 - DNA, 63 bp, synthetic construct; identical to SEQ ID NO: 1
  source 1..63: mol_type = other DNA

SEQ ID NO: 114 - DNA, 366 bp, synthetic construct; identical to SEQ ID NO: 7
  source 1..366: mol_type = other DNA

SEQ ID NO: 115 - DNA, 54 bp, synthetic construct; identical to SEQ ID NO: 5
  source 1..54: mol_type = other DNA

SEQ ID NO: 116 - DNA, 321 bp, synthetic construct; identical to SEQ ID NO: 3
  source 1..321: mol_type = other DNA

SEQ ID NO: 117 - DNA, 15 bp, synthetic construct
  source 1..15: mol_type = other DNA
ggaggtggtggatcc

SEQ ID NO: 118 - DNA, 363 bp, synthetic construct; identical to SEQ ID NO: 15
  source 1..363: mol_type = other DNA

SEQ ID NO: 119 - DNA, 45 bp, synthetic construct; identical to SEQ ID NO: 13
  source 1..45: mol_type = other DNA

SEQ ID NO: 120 - DNA, 321 bp, synthetic construct; identical to SEQ ID NO: 11
  source 1..321: mol_type = other DNA

SEQ ID NO: 121 - DNA, 36 bp, synthetic construct; identical to SEQ ID NO: 77
  source 1..36: mol_type = other DNA

SEQ ID NO: 122 - DNA, 84 bp, synthetic construct; identical to SEQ ID NO: 79
  source 1..84: mol_type = other DNA

SEQ ID NO: 123 - DNA, 126 bp, synthetic construct; identical to SEQ ID NO: 21
  source 1..126: mol_type = other DNA

SEQ ID NO: 124 - DNA, 336 bp, synthetic construct; identical to SEQ ID NO: 82
  source 1..336: mol_type = other DNA

SEQ ID NO: 125 - DNA, 2133 bp, synthetic construct
  source 1..2133: mol_type = other DNA
atggccttaccagtgaccgccttgctcctgccgctggccttgctgctccacgccgccaggccggaagtgcagctggtggagtctgggggaggcttggtacagcctggcaggtccctgagactctcctgtgcagcctctggattcacctttaatgattatgccatgcactgggtccggcaagctccagggaagggcctggagtgggtctcaactattagttggaatagtggttccataggctatgcggactctgtgaagggccgattcaccatctccagagacaacgccaagaagtccctgtatctgcaaatgaacagtctgagagctgaggacacggccttgtattactgtgcaaaagatatacagtacggcaactactactacggtatggacgtctggggccaagggaccacggtcaccgtctcctcaggcagtactagcggtggtggctccgggggcggttccggtgggggcggcagcagcgaaattgtgttgacacagtctccagccaccctgtctttgtctccaggggaaagagccaccctctcctgcagggccagtcagagtgttagcagctacttagcctggtaccaacagaaacctggccaggctcccaggctcctcatctatgatgcatccaacagggccactggcatcccagccaggttcagtggcagtgggtctgggacagacttcactctcaccatcagcagcctagagcctgaagattttgcagtttattactgtcagcagcgtagcaactggccgatcaccttcggccaagggacacgactggagattaaaggaggtggtggatccgaggtgcagctggtggagtccggcggcggcctggtgcagcccggcggctccctgcggctgtcctgcgccgcctccggcttcaccttctccaacttcgacatggcctgggtgcggcaggcccccggcaagggcctggtgtgggtgtcctccatcaccaccggcgccgaccacgccatctacgccgactccgtgaagggccggttcaccatctcccgggacaacgccaagaacaccctgtacctgcagatgaactccctgcgggccgaggacaccgccgtgtactactgcgtgcggcacggctactacgacggctaccacctgttcgactactggggccagggcaccctggtgaccgtgtcctccggtggcggtggctcgggcggtggtgggtcgggtggcggcggatctgacatccagatgacccagtccccctcctccctgtccgcctccgtgggcgaccgggtgaccatcacctgccgggcctcccagggcatctccaactacctgaactggtaccagcagaagcccggcaaggcccccaagcccctgatctactacacctccaacctgcagtccggcgtgccctcccggttctccggctccggctccggcaccgactacaccctgaccatctcctccctgcagcccgaggacttcgccacctactactgcatgggccagaccatctcctcctacaccttcggccagggcaccaagctggagatcaaggagagcaagtacggaccgccctgccccccttgccctatgttctgggtgctggtggtggtcggaggcgtgctggcctgctacagcctgctggtcaccgtggccttcatcatcttttgggtgaaacggggcagaaagaaactcctgtatatattcaaacaaccatttatgagaccagtacaaactactcaagaggaagatggctgtagctgccgatttccagaagaagaagaaggaggatgtgaactgcgggtgaagttcagcagaagcgccgacgcccctgcctaccagcagggccagaatcagctgtacaacgagctgaacctgggcagaagggaagagtacgacgtcctggataagcggagaggccgggaccctgagatgggcggcaagcctcggcggaagaacccccaggaaggcctgtataacgaactgcagaaagacaagatggccgaggcctacagcgagatcggcatgaagggcgagcggaggcggggcaagggccacgacggcctgtatcagggcctgtccaccgccaccaaggatacctacgacgccctgcacatgcaggccctgcccccaaggtaa

SEQ ID NO: 126 - protein, 710 aa, synthetic construct
MALPVTALLLPLALLLHAARPEVQLVESGGGLVQPGRSLRLSCAASGFTFNDYAMHWVRQAPGKGLEWVSTISWNSGSIGYADSVKGRFTISRDNAKKSLYLQMNSLRAEDTALYYCAKDIQYGNYYYGMDVWGQGTTVTVSSGSTSGGGSGGGSGGGGSSEIVLTQSPATLSLSPGERATLSCRASQSVSSYLAWYQQKPGQAPRLLIYDASNRATGIPARFSGSGSGTDFTLTISSLEPEDFAVYYCQQRSNWPITFGQGTRLEIKGGGGSEVQLVESGGGLVQPGGSLRLSCAASGFTFSNFDMAWVRQAPGKGLVWVSSITTGADHAIYADSVKGRFTISRDNAKNTLYLQMNSLRAEDTAVYYCVRHGYYDGYHLFDYWGQGTLVTVSSGGGGSGGGGSGGGGSDIQMTQSPSSLSASVGDRVTITCRASQGISNYLNWYQQKPGKAPKPLIYYTSNLQSGVPSRFSGSGSGTDYTLTISSLQPEDFATYYCMGQTISSYTFGQGTKLEIKESKYGPPCPPCPMFWVLVVVGGVLACYSLLVTVAFIIFWVKRGRKKLLYIFKQPFMRPVQTTQEEDGCSCRFPEEEEGGCELRVKFSRSADAPAYQQGQNQLYNELNLGRREEYDVLDKRRGRDPEMGGKPRRKNPQEGLYNELQKDKMAEAYSEIGMKGERRRGKGHDGLYQGLSTATKDTYDALHMQALPPR

SEQ ID NO: 127 - protein, 6 aa, synthetic construct
NDYAMH

SEQ ID NO: 128 - protein, 17 aa, synthetic construct
TISWNSGSIGYADSVKG

SEQ ID NO: 129 - protein, 13 aa, synthetic construct
DIQYGNYYYGMDV

SEQ ID NO: 130 - protein, 11 aa, synthetic construct
RASQSVSSYLA

SEQ ID NO: 131 - protein, 7 aa, synthetic construct
DASNRAT

SEQ ID NO: 132 - protein, 9 aa, synthetic construct
QQRSNWPIT

SEQ ID NO: 133 - protein, 23 aa, synthetic construct
DIQMTQSPSSLSASVGDRVTITC

SEQ ID NO: 134 - protein, 11 aa, synthetic construct
RASQGISNYLN

SEQ ID NO: 135 - protein, 15 aa, synthetic construct
WYQQKPGKAPKPLIY

SEQ ID NO: 136 - protein, 7 aa, synthetic construct
YTSNLQS

SEQ ID NO: 137 - protein, 32 aa, synthetic construct
GVPSRFSGSGSGTDYTLTISSLQPEDFATYYC

SEQ ID NO: 138 - protein, 9 aa, synthetic construct
MGQTISSYT

SEQ ID NO: 139 - protein, 10 aa, synthetic construct
FGQGTKLEIK

SEQ ID NO: 140 - protein, 30 aa, synthetic construct
EVQLVESGGGLVQPGGSLRLSCAASGFTFS

SEQ ID NO: 141 - protein, 5 aa, synthetic construct
NFDMA

SEQ ID NO: 142 - protein, 14 aa, synthetic construct
WVRQAPGKGLVWVS

SEQ ID NO: 143 - protein, 17 aa, synthetic construct
SITTGADHAIYADSVKG

SEQ ID NO: 144 - protein, 32 aa, synthetic construct
RFTISRDNAKNTLYLQMNSLRAEDTAVYYCVR

SEQ ID NO: 145 - protein, 12 aa, synthetic construct
HGYYDGYHLFDY

SEQ ID NO: 146 - protein, 11 aa, synthetic construct
WGQGTLVTVSS